European Patent Application EP 4 481 043 A1, published December 25, 2024. Title: APTAMER FOR SPECIFICALLY RECOGNIZING SOLUBLE ST2 PROTEIN AND APPLICATION OF THE SAME. Applicant: Beijing Institute of Heart, Lung and Blood Vessel Diseases. Application US. The sequence listing filed with the application follows.

SEQUENCE LISTING (13 sequences)

SEQ ID NO: 1 - DNA, 35 bp, synthetic construct
  source 1..35: mol_type = other DNA
tccatccactcggggctagaagccgtgagaatctg

SEQ ID NO: 2 - DNA, 35 bp, synthetic construct
  source 1..35: mol_type = other DNA
tccatccactcgggccctagggcgtgtatgtccat

SEQ ID NO: 3 - DNA, 35 bp, synthetic construct
  source 1..35: mol_type = other DNA
tccatccactcggcctactaagggtttcgttcacc

SEQ ID NO: 4 - DNA, 36 bp, synthetic construct
  source 1..36: mol_type = other DNA
tccatccactcggggcgggggctcgtgctctatttc

SEQ ID NO: 5 - DNA, 35 bp, synthetic construct
  source 1..35: mol_type = other DNA
cctccatccactcggcgcaacgccggggctcggcc

SEQ ID NO: 6 - DNA, 35 bp, synthetic construct
  source 1..35: mol_type = other DNA
tccattcactcgaccgctgacgcgggtgtcgtttt

SEQ ID NO: 7 - DNA, 35 bp, synthetic construct
  source 1..35: mol_type = other DNA
tccatgcactcgcccttgaaagggttccctccgtt

SEQ ID NO: 8 - DNA, 35 bp, synthetic construct
  source 1..35: mol_type = other DNA
tccatccactcggcgccacgcggtttctccagatt

SEQ ID NO: 9 - DNA, 35 bp, synthetic construct
  source 1..35: mol_type = other DNA
tccatgcactcgcgctaccggcgtgcccgtagatc

SEQ ID NO: 10 - DNA, 35 bp, synthetic construct
  source 1..35: mol_type = other DNA
tccattcactcgcagcggggtcgcgtgaggcgcaa

SEQ ID NO: 11 - DNA, 75 bp, synthetic construct
  source 1..75: mol_type = other DNA
gacaggcaggacaccgtaacnnnnnnnnnnnnnnnnnnnnnnnnnnnnnnnnnnnctgctacctccctcctcttc

SEQ ID NO: 12 - DNA, 20 bp, synthetic construct
  source 1..20: mol_type = other DNA
gacaggcaggacaccgtaac

SEQ ID NO: 13 - DNA, 20 bp, synthetic construct
  source 1..20: mol_type = other DNA
gaagaggagggaggtagcag